European Patent Specification EP 3 329 037 B1, published October 18, 2023. Title: STABLE PROTEINS AND METHODS FOR DESIGNING SAME. Applicant: Yeda Research And Development Co. Ltd. FLEISHMAN, Sarel GOLDENZWEIG, Adi TAWFIK, Dan S. The sequence listing filed with the application follows.

SEQUENCE LISTING (11 sequences)

SEQ ID NO: 1 - protein, 542 aa, Homo sapiens
GREDAELLVTVRGGRLRGIRLKTPGGPVSAFLGIPFAEPPMGPRRFLPPEPKQPWSGVVDATTFQSVCYQYVDTLYPGFEGTEMWNPNRELSEDCLYLNVWTPYPRPTSPTPVLVWIYGGGFYSGASSLDVYDGRFLVQAERTVLVSMNYRVGAFGFLALPGSREAPGNVGLLDQRLALQWVQENVAAFGGDPTSVTLFGESAGAASVGMHLLSPPSRGLFHRAVLQSGAPNGPWATVGMGEARRRATQLAHLVGCPPGGTGGNDTELVACLRTRPAQVLVNHEWHVLPQESVFRFSFVPVVDGDFLSDTPEALINAGDFHGLQVLVGVVKDEGSYFLVYGAPGFSKDNESLISRAEFLAGVRVGVPQVSDLAAEAVVLHYTDWLHPEDPARLREALSDVVGDHNVVCPVAQLAGRLAAQGARVYAYVFEHRASTLSWPLWMGVPHGYEIEFIFGIPLDPSRNYTAEEKIFAQRLMRYWANFARTGDPNEPRDPKAPQWPPYTAGAQQYVSLDLRPLEVRRGLRAQACAFWNRFLPKLLSAT

SEQ ID NO: 2 - protein, 544 aa, Artificial sequence
  Amino Acid sequence encoding RhAChE_m0p9
MEGREDAELLVTTRGGRLRGIRLMTPGGPVSAFLGIPFAEPPVGPRRFRPPEPKQPWSGVWDATTFQNVCYQYVDTLYPGFEGTEMWNPNRNLSEDCLYLNVWTPYPRPKNPAPVMVWIYGGGFYSGSSSLDVYDGRFLVRTERVVLVSMNYRVGAFGFLALPGSREAPGNVGLLDQRLALQWVQENIAAFGGDPTSVTLFGESAGAASVGMHLLSPPSRGLFHRAILQSGAPNAPWATVSMEEARRRATQLAKLVGCPPGGTGGNDTELVACLRTRPPQELVNHEWHVLPQESVFRFSFVPVVDGDFLPDTPEALINNGDFKGLDVLVGVNKDEGSYFLVYGAPGFSKDNESLISREEFLAGVRVGVPQVSDLAAEAVVLHYTDWLHPEDPARLREALSDVVGDHNVICPVAQFAQRYAANGARVYMYVFEHRSSTLPWPEWMGVPHGYEIEFIFGIPLDPSRNYTEEEKIFARRLMRYWANFARTGDPNEPRDPKAPQWPPYTADAQKYVSLDLRPLEVRRGLRAQACAFWNRFLPKLLSAT

SEQ ID NO: 3 - protein, 544 aa, Artificial sequence
  Amino Acid sequence encoding RhAChE_m0p45
MEGREDAELIVTTRGGKIRGIRLTTIGGPVSAFLGIPFAEPPVGPRRFRPPEPKRPWSGVWDATTFQNVCYQYVDTLYPGFPGTEMWNPNRPLSEDCLYLNVWTPYPRPKNPAPVMVWIYGGGFYSGSSSLDVYDGRFLVREERVVLVSMNYRVGAFGFLALPGSREAPGNVGLLDQRLALQWVQENIAAFGGDPTNVTLFGESAGAASVGMHLLSPPSRGLFHRAILQSGAPNAPWAYVSREEARRRALQLAKLVGCPPGGTGGNDTELVACLRNRPAQELVNHEWHVLPQESVFRFSFVPVVDGSFLPDTPEALINNGDFKGLQVLVGVNKDEGSYFLVYGAPGFSKDNESLISREEFLEGVRVGVPNVSDLAAEAIVLHYTDWLHPDDPEKNRDALADVVGDHNVICPVAQFAERYAANGARVYAYFFEHRSSTLPWPEWMGVPHGYEIEFVFGIPLDPSKNYTKEEKIFARRMMRYWANFARTGDPNEPRDPKAPQWPPYTADEQKYVSLDLRPLEVRRGLRAQHCAFWNRFLPKLLSMT

SEQ ID NO: 4 - protein, 544 aa, Artificial sequence
  Amino Acid sequence encoding RhAChE_m0p7
MEGREDAELLVTTRGGRLRGIRLTTPGGPVSAFLGIPFAEPPVGPRRFRPPEPKQPWSGVWDATTFQNVCYQYVDTLYPGFEGTEMWNPNRNLSEDCLYLNVWTPYPRPKNPAPVMVWIYGGGFYSGSSSLDVYDGRFLVRTERVVLVSMNYRVGAFGFLALPGSREAPGNVGLLDQRLALQWVQENIAAFGGDPTSVTLFGESAGAASVGMHLLSPPSRGLFHRAILQSGAPNAPWAYVSREEARRRALQLAKLVGCPPGGTGGNDTELVACLRNRPPQELVNHEWHVLPQESVFRFSFVPVVDGDFLPDTPEALINNGDFKGLDVLVGVNKDEGSYFLVYGAPGFSKDNESLISREEFLEGVRVGVPQVSDLAAEAIVLHYTDWLHPEDPAKNRDALSDVVGDHNVICPVAQFAQRYAANGARVYAYVFEHRSSTLPWPEWMGVPHGYEIEFIFGIPLDPSRNYTKEEKIFARRLMRYWANFARTGDPNEPRDPKAPQWPPYTADEQKYVSLDLRPLEVRRGLRAQACAFWNRFLPKLLSAT

SEQ ID NO: 5 - protein, 544 aa, Artificial sequence
  Amino Acid sequence encoding RhAChE_m1p2
MEGREDAELLVTTRGGRLRGIRLKTPGGPVSAFLGIPFAEPPVGPRRFRPPEPKQPWSGVWDATTFQNVCYQYVDTLYPGFEGTEMWNPNRELSEDCLYLNVWTPYPRPTSPVPVMVWIYGGGFYSGSSSLDVYDGRFLVRAERVVLVSMNYRVGAFGFLALPGSREAPGNVGLLDQRLALQWVQENIAAFGGDPTSVTLFGESAGAASVGMHLLSPPSRGLFHRAILQSGAPNAPWATVSMEEARRRATQLAKLVGCPPGGTGGNDTELVACLRTRPPQVLVNHEWHVLPQESVFRFSFVPVVDGDFLPDTPEALINNGDFKGLQVLVGVNKDEGSYFLVYGAPGFSKDNESLISREEFLAGVRVGVPQVSDLAAEAVVLHYTDWLHPEDPARLREALSDVVGDHNVVCPVAQFAQRYAAQGARVYMYVFEHRASTLPWPEWMGVPHGYEIEFIFGIPLDPSRNYTAEEKIFAQRLMRYWANFARTGDPNEPRDPKAPQWPPYTADAQQYVSLDLRPLEVRRGLRAQHCAFWNRFLPKLLSAT

SEQ ID NO: 6 - protein, 544 aa, Artificial sequence
  Amino Acid sequence encoding RhAChE_m2p0
MEGREDAELLVTVRGGRLRGIRLKTPGGPVSAFLGIPFAEPPMGPRRFRPPEPKQPWSGVWDATTFQNVCYQYVDTLYPGFEGTEMWNPNRELSEDCLYLNVWTPYPRPTSPTPVMVWIYGGGFYSGSSSLDVYDGRFLVQAERVVLVSMNYRVGAFGFLALPGSREAPGNVGLLDQRLALQWVQENIAAFGGDPTSVTLFGESAGAASVGMHLLSPPSRGLFHRAILQSGAPNAPWATVSMGEARRRATQLAKLVGCPPGGTGGNDTELVACLRTRPAQVLVNHEWHVLPQESVFRFSFVPVVDGDFLSDTPEALINAGDFHGLQVLVGVNKDEGSYFLVYGAPGFSKDNESLISRAEFLAGVRVGVPQVSDLAAEAVVLHYTDWLHPEDPARLREALSDVVGDHNVVCPVAQFAQRYAAQGARVYAYVFEHRASTLPWPEWMGVPHGYEIEFIFGIPLDPSRNYTAEEKIFAQRLMRYWANFARTGDPNEPRDPKAPQWPPYTAGAQQYVSLDLRPLEVRRGLRAQACAFWNRFLPKLLSAT

SEQ ID NO: 7 - protein, 342 aa, Artificial sequence
  Amino Acid sequence encoding PTE-S5  variant of PTE
GRISEFITNSGDRINTVRGPITISEAGFTLTHEHICGSSAGFLRAWPEFFGSRKALAEKAVRGLRRARAAGVRTIVDVSTFDIGRDVSLLAEVSRAADVHIVAATGLWFDPPLSMRLRSVEELTQFFLREIQYGIEDTGIRAGIIKVATTGKATPFQELVLRAAARASLATGVPVTTHTAASQRGGEQQAAIFESEGLSPSRVCIGHSDDTDDLSYLTALAARGYLIGLDHIPHSAIGLEDNASASALLGIRSWQTRALLIKALIDQGYMKQILVSNDWLFGFSSYVTNIMDVMDSVNPDGMAFIPLRVIPFLREKGVPQETLAGITVTNPARFLSPTLRAS

SEQ ID NO: 8 - protein, 342 aa, Artificial sequence
  Amino Acid sequence encoding dPTE_m0p45
GRISEFITNSGDRINTVRGPITISELGFTLMHEHICGSSAGFLRAWPEFFGSRDALAEKAVRGLRRARAAGVDTIVDVSTFDIGRDVELLAEVAEAADVHIVAATGLWFDPPLSMRLRSVEELTQFFLREIQYGIEDTGIRAGIIKVATTGKATPFQERVLRAAARASLETGVPVTTHTDASQRDGEEQADIFESEGLDPSRVCIGHADDTDDLDYLTELAARGYLIGLDHIPHSAIGLEDNASAAALLGLRSWQTRALLIKALIDQGYADQILVSNDWLFGFSSYVTNIMDVMDRVNPDGMAHIPERVIPFLREKGVPDETLDTIMVENPARFLSPTLRAS

SEQ ID NO: 9 - protein, 342 aa, Artificial sequence
  Amino Acid sequence encoding dPTE_m1p00
GRISEFITNSGDRINTVRGPITISEAGFTLMHEHICGSSAGFLRAWPEFFGSRDALAEKAVRGLRRARAAGVRTIVDVSTFDIGRDVELLAEVSEAADVHIVAATGLWFDPPLSMRLRSVEELTQFFLREIQYGIEDTGIRAGIIKVATTGKATPFQERVLRAAARASLATGVPVTTHTDASQRDGEQQADIFESEGLDPSRVCIGHSDDTDDLDYLTALAARGYLIGLDHIPHSAIGLEDNASAAALLGLRSWQTRALLIKALIDQGYADQILVSNDWLFGFSSYVTNIMDVMDRVNPDGMAFIPLRVIPFLREKGVPDETLETIMVDNPARFLSPTLRAS

SEQ ID NO: 10 - protein, 342 aa, Artificial sequence
  Amino Acid sequence encoding dPTE_m2p00
GRISEFITNSGDRINTVRGPITISEAGFTLTHEHICGSSAGFLRAWPEFFGSRDALAEKAVRGLRRARAAGVRTIVDVSTFDIGRDVSLLAEVSEAADVHIVAATGLWFDPPLSMRLRSVEELTQFFLREIQYGIEDTGIRAGIIKVATTGKATPFQELVLRAAARASLATGVPVTTHTDASQRDGEQQAAIFESEGLDPSRVCIGHSDDTDDLDYLTALAARGYLIGLDHIPHSAIGLEDNASASALLGIRSWQTRALLIKALIDQGYVKQILVSNDWLFGFSSYVTNIMDVMDRVNPDGMAFIPLRVIPFLREKGVPQETLATITVENPARFLSPTLRAS

SEQ ID NO: 11 - protein, 287 aa, Artificial sequence
  Amino Acid sequence encoding Dnmt3a_Stab
MPAEKRKPIRVLSLFDGIATGLLVLKDLGIQVDRYIASEVCEDSITVGMVRHQGNIMYVGDVRNITQKHIDEWGPFDLVIGGSPCNDLSIVNPARKGLYEGTGRLFFEFYRLLHDARPKEGDDRPFFWLFENVVAMRVNDKRDISRFLECNPVMIDAKEVSAAHRARYFWGNLPGMNRPLCPSKNDKLELQECLEHGRQAKFSKVRTITTRSNSIKQGKDQHFPVFMNGKEDILWCTEMERVFGFPDHYTDVSNMSRLARQRLLGRSWSVPVIRHLFAPLKDYFACV